European Patent Application EP 4 477 661 A1, published December 18, 2024. Title: LONG-LASTING HEPATITIS VIRUS ENTRY INHIBITOR. Applicant: CHENGDU AODA BIOTECHNOLOGY CO., LTD. Application CN PCT/CN2022/136263, filed December 2, 2022. The sequence listing filed with the application follows.

SEQUENCE LISTING (43 sequences)

SEQ ID NO: 1 - protein, 47 aa, synthetic construct
  MOD_RES 1: note = eicosanedioic acid-gamma Glu-modified Gly
  MOD_RES 47: note = NH2-modified Gly
GTNLSVPNPLGFFPDHQLDPAFGANSNNPDWDFNPNKDHWPEANKVG

SEQ ID NO: 2 - protein, 47 aa, synthetic construct; identical to SEQ ID NO: 1
  MOD_RES 1: note = eicosandioic acid-gamma Glu-PEG1CH2CO- modified Gly
  MOD_RES 47: note = NH2-modified Gly

SEQ ID NO: 3 - protein, 47 aa, synthetic construct; identical to SEQ ID NO: 1
  MOD_RES 47: note = Eicosanedioic acid -gamma Glu-PEG2CH2CO- modified Gly
  MOD_RES 47: note = -NH2-modified Gly

SEQ ID NO: 4 - protein, 47 aa, synthetic construct; identical to SEQ ID NO: 1
  MOD_RES 47: note = Eicosanedioic acid -gamma Glu-PEG3CH2CO- modified Gly
  MOD_RES 47: note = -NH2-modified Gly

SEQ ID NO: 5 - protein, 47 aa, synthetic construct; identical to SEQ ID NO: 1
  MOD_RES 47: note = Eicosanedioic acid -gamma Glu-PEG4CH2CO- modified Gly
  MOD_RES 47: note = -NH2-modified Gly

SEQ ID NO: 6 - protein, 47 aa, synthetic construct; identical to SEQ ID NO: 1
  MOD_RES 47: note = Eicosanedioic acid -gamma Glu-PEG5CH2CO- modified Gly
  MOD_RES 47: note = NH2-modified Gly

SEQ ID NO: 7 - protein, 47 aa, synthetic construct; identical to SEQ ID NO: 1
  MOD_RES 47: note = Eicosanedioic acid -gamma Glu-PEG6CH2CO- modified Gly
  MOD_RES 47: note = -NH2-modified Gly

SEQ ID NO: 8 - protein, 47 aa, synthetic construct; identical to SEQ ID NO: 1
  MOD_RES 47: note = Eicosanedioic acid -gamma Glu-Gly- modified Gly
  MOD_RES 47: note = -NH2-modified Gly

SEQ ID NO: 9 - protein, 47 aa, synthetic construct; identical to SEQ ID NO: 1
  MOD_RES 47: note = Eicosanedioic acid -gamma Glu-Gly-Gly-modified Gly
  MOD_RES 47: note = -NH2-modified Gly

SEQ ID NO: 10 - protein, 47 aa, synthetic construct; identical to SEQ ID NO: 1
  MOD_RES 47: note = Eicosanedioic acid -gamma Glu-Gly-Gly-Gly- modified Gly
  MOD_RES 47: note = -NH2-modified Gly

SEQ ID NO: 11 - protein, 47 aa, synthetic construct; identical to SEQ ID NO: 1
  MOD_RES 47: note = Eicosanedioic acid -gamma Glu-Gly-Gly-Gly-Gly- modified Gly
  MOD_RES 47: note = -NH2-modified Gly

SEQ ID NO: 12 - protein, 47 aa, synthetic construct; identical to SEQ ID NO: 1
  MOD_RES 47: note = Eicosanedioic acid -gamma Glu- Gly-Gly-Gly-Gly- modified Gly
  MOD_RES 47: note = -NH2-modified Gly

SEQ ID NO: 13 - protein, 47 aa, synthetic construct; identical to SEQ ID NO: 1
  MOD_RES 47: note = Eicosanedioic acid -gamma Glu- Gly-Gly-Gly-Gly-Gly-Gly-Gly- modified Gly
  MOD_RES 47: note = -NH2-modified Gly

SEQ ID NO: 14 - protein, 47 aa, synthetic construct; identical to SEQ ID NO: 1
  MOD_RES 47: note = Eicosanedioic acid -gamma Glu- Gly-Gly-Ser-Gly-Ser-Gly- modified Gly
  MOD_RES 47: note = -NH2-modified Gly

SEQ ID NO: 15 - protein, 47 aa, synthetic construct
  MOD_RES 47: note = Eicosanedioic acid -gamma Glu- modified Gly
  MOD_RES 47: note = -NH2-modified Gly
GTNLSVPNPLGFFPDHQLDPAFGANSNNPDWDFNPNKDHWPEANRVG

SEQ ID NO: 16 - protein, 47 aa, synthetic construct; identical to SEQ ID NO: 15
  MOD_RES 47: note = Eicosanedioic acid -gamma Glu-PEG1CH2CO- modified Gly
  MOD_RES 47: note = -NH2-modified Gly

SEQ ID NO: 17 - protein, 47 aa, synthetic construct; identical to SEQ ID NO: 15
  MOD_RES 47: note = Eicosanedioic acid -gamma Glu-PEG2CH2CO- modified Gly
  MOD_RES 47: note = -NH2-modified Gly

SEQ ID NO: 18 - protein, 47 aa, synthetic construct; identical to SEQ ID NO: 15
  MOD_RES 47: note = Eicosanedioic acid -gamma Glu-PEG3CH2CO- modified Gly
  MOD_RES 47: note = -NH2-modified Gly

SEQ ID NO: 19 - protein, 47 aa, synthetic construct; identical to SEQ ID NO: 15
  MOD_RES 47: note = Eicosanedioic acid -gamma Glu-PEG4CH2CO- modified Gly
  MOD_RES 47: note = -NH2-modified Gly

SEQ ID NO: 20 - protein, 47 aa, synthetic construct; identical to SEQ ID NO: 15
  MOD_RES 47: note = Eicosanedioic acid -gamma Glu-PEG5CH2CO- modified Gly
  MOD_RES 47: note = -NH2-modified Gly

SEQ ID NO: 21 - protein, 47 aa, synthetic construct; identical to SEQ ID NO: 15
  MOD_RES 47: note = Eicosanedioic acid -gamma Glu-PEG6CH2CO- modified Gly
  MOD_RES 47: note = -NH2-modified Gly

SEQ ID NO: 22 - protein, 47 aa, synthetic construct; identical to SEQ ID NO: 15
  MOD_RES 47: note = Eicosanedioic acid -gamma Glu-Gly- modified Gly
  MOD_RES 47: note = -NH2-modified Gly

SEQ ID NO: 23 - protein, 47 aa, synthetic construct; identical to SEQ ID NO: 15
  MOD_RES 47: note = Eicosanedioic acid -gamma Glu-Gly-Gly- modified Gly
  MOD_RES 47: note = -NH2-modified Gly

SEQ ID NO: 24 - protein, 47 aa, synthetic construct; identical to SEQ ID NO: 15
  MOD_RES 47: note = Eicosanedioic acid -gamma Glu-Gly-Gly-Gly- modified Gly
  MOD_RES 47: note = -NH2-modified Gly

SEQ ID NO: 25 - protein, 47 aa, synthetic construct; identical to SEQ ID NO: 15
  MOD_RES 47: note = Eicosanedioic acid -gamma Glu-Gly-Gly-Gly-Gly- modified Gly
  MOD_RES 47: note = -NH2-modified Gly

SEQ ID NO: 26 - protein, 47 aa, synthetic construct; identical to SEQ ID NO: 15
  MOD_RES 47: note = Eicosanedioic acid -gamma Glu-Gly-Gly-Gly-Gly- modified Gly
  MOD_RES 47: note = -NH2-modified Gly

SEQ ID NO: 27 - protein, 47 aa, synthetic construct; identical to SEQ ID NO: 15
  MOD_RES 47: note = Eicosanedioic acid -gamma Glu-Gly-Gly-Gly-Gly-Gly-Gly- modified Gly
  MOD_RES 47: note = -NH2-modified Gly

SEQ ID NO: 28 - protein, 47 aa, synthetic construct; identical to SEQ ID NO: 15
  MOD_RES 47: note = Eicosanedioic acid-gamma Glu-Gly-Gly-Ser-Gly-Ser-Gly-modified Gly
  MOD_RES 47: note = -NH2-modified Gly

SEQ ID NO: 29 - protein, 47 aa, synthetic construct
  MOD_RES 47: note = Eicosanedioic acid-gamma Glu-Gly-Thr-Asn-Leu-Ser-Val-Pro-Asn- Pro-Leu-modified Gly
  MOD_RES 47: note = -NH2-modified Gly
GTNLSVPNPLGFFPDHQLDPAFGANSNNPDWDFNPNKDHWPEANQVG

SEQ ID NO: 30 - protein, 47 aa, synthetic construct; identical to SEQ ID NO: 29
  MOD_RES 47: note = Eicosanedioic acid-gamma Glu-PEG1CH2CO-modified Gly
  MOD_RES 47: note = -NH2-modified Gly

SEQ ID NO: 31 - protein, 47 aa, synthetic construct; identical to SEQ ID NO: 29
  MOD_RES 47: note = Eicosanedioic acid-gamma Glu-PEG2CH2CO-modified Gly
  MOD_RES 47: note = -NH2-modified Gly

SEQ ID NO: 32 - protein, 47 aa, synthetic construct; identical to SEQ ID NO: 29
  MOD_RES 47: note = Eicosanedioic acid-gamma Glu-PEG3CH2CO-modified Gly
  MOD_RES 47: note = -NH2-modified Gly

SEQ ID NO: 33 - protein, 47 aa, synthetic construct; identical to SEQ ID NO: 29
  MOD_RES 47: note = Eicosanedioic acid-gamma Glu-PEG4CH2CO-modified Gly
  MOD_RES 47: note = -NH2-modified Gly

SEQ ID NO: 34 - protein, 47 aa, synthetic construct; identical to SEQ ID NO: 29
  MOD_RES 47: note = Eicosanedioic acid-gamma Glu-PEG5CH2CO-modified Gly
  MOD_RES 47: note = -NH2-modified Gly

SEQ ID NO: 35 - protein, 47 aa, synthetic construct; identical to SEQ ID NO: 29
  MOD_RES 47: note = -NH2-modified Gly
  MOD_RES 47: note = Eicosanedioic acid-gamma Glu-PEG6CH2CO-modified G

SEQ ID NO: 36 - protein, 47 aa, synthetic construct; identical to SEQ ID NO: 29
  MOD_RES 47: note = Eicosanedioic acid-gamma Glu-Gly-modified Gly
  MOD_RES 47: note = -NH2-modified Gly

SEQ ID NO: 37 - protein, 47 aa, synthetic construct; identical to SEQ ID NO: 29
  MOD_RES 47: note = Eicosanedioic acid-gamma Glu-Gly-Gly-modified Gly
  MOD_RES 47: note = -NH2-modified Gly

SEQ ID NO: 38 - protein, 47 aa, synthetic construct; identical to SEQ ID NO: 29
  MOD_RES 47: note = Eicosanedioic acid-gamma Glu-Gly-Gly-Gly-modified Gly
  MOD_RES 47: note = -NH2-modified Gly

SEQ ID NO: 39 - protein, 47 aa, synthetic construct; identical to SEQ ID NO: 29
  MOD_RES 47: note = Eicosanedioic acid-gamma Glu-Gly-Gly-Gly-Gly-modified Gly
  MOD_RES 47: note = -NH2-modified Gly

SEQ ID NO: 40 - protein, 47 aa, synthetic construct; identical to SEQ ID NO: 29
  MOD_RES 47: note = Eicosanedioic acid-gamma Glu-Gly-Gly-Gly-Gly-Gly-modified Gly
  MOD_RES 47: note = -NH2-modified Gly

SEQ ID NO: 41 - protein, 47 aa, synthetic construct; identical to SEQ ID NO: 29
  MOD_RES 47: note = Eicosanedioic acid-gamma Glu-Gly-Gly-Gly-Gly-Gly-Gly- modified Gly
  MOD_RES 47: note = -NH2-modified Gly

SEQ ID NO: 42 - protein, 47 aa, synthetic construct; identical to SEQ ID NO: 29
  MOD_RES 47: note = Eicosanedioic acid-gamma Glu-Gly-Gly-Ser-Gly-Ser-Gly-modified Gly
  MOD_RES 47: note = -NH2-modified Gly

SEQ ID NO: 43 - protein, 47 aa, synthetic construct
  MOD_RES 47: note = HO2C(CH2)n1CO-(AA3)n2-(PEGn3(CH2)n4CO)n5-modified Gly, or HO2C(CH2)n1CO-(AA3)n2-(AA4)n6-modified Gly; wherein: n1 is an integer selected from 10 to 20; n2 is an integer selected from 1 to 5; n3 is an integer selected from 1 to 30; n4 is an integer; n5 is 0, or an integer selected from 1 to 5; n6 is 0, or an integer selected from 1 to 10; AA3 is gamma Glu, epsilon Lys, beta Ala, gamma aminobutyric acid, or 5-Ava. AA4 is Ala, Gly,Leu, Ser, Thr, Tyr, Gln, Lys, Dao, Dah, Orn, Dab, Dap, Glu, Asp, Ada, Apm, or Asu.
  MOD_RES 47: note = -NH2-modified Gly, or -OH-modified Gly.
GTNLSVPNPLGFFPDHQLDPAFGANSNNPDWDFNPNKDHWPEANXVG